European Patent Specification EP 3 430 030 B1, published December 20, 2023. Title: TRANSFECTED T-CELLS AND T-CELL RECEPTORS FOR USE IN IMMUNOTHERAPY AGAINST CANCERS. Applicant: Immatics Biotechnologies GmbH. The sequence listing filed with the application follows.

SEQUENCE LISTING (101 sequences)

SEQ ID NO: 1 - protein, 9 aa, Homo sapiens
KVLEHVVRV

SEQ ID NO: 2 - protein, 9 aa, Homo sapiens
KVLEHVVRL

SEQ ID NO: 3 - protein, 9 aa, Homo sapiens
KVLEHVVRA

SEQ ID NO: 4 - protein, 9 aa, Homo sapiens
KVLEHVVRI

SEQ ID NO: 5 - protein, 9 aa, Homo sapiens
KLLEHVVRV

SEQ ID NO: 6 - protein, 9 aa, Homo sapiens
KLLEHVVRL

SEQ ID NO: 7 - protein, 9 aa, Homo sapiens
KLLEHVVRA

SEQ ID NO: 8 - protein, 9 aa, Homo sapiens
KLLEHVVRI

SEQ ID NO: 9 - protein, 9 aa, Homo sapiens
KALEHVVRV

SEQ ID NO: 10 - protein, 9 aa, Homo sapiens
KALEHVVRL

SEQ ID NO: 11 - protein, 9 aa, Homo sapiens
KALEHVVRA

SEQ ID NO: 12 - protein, 9 aa, Homo sapiens
KALEHVVRI

SEQ ID NO: 13 - protein, 9 aa, Homo sapiens
YLLEHVVRV

SEQ ID NO: 14 - protein, 9 aa, Homo sapiens
YLLEHVVRL

SEQ ID NO: 15 - protein, 9 aa, Homo sapiens
YLLEHVVRA

SEQ ID NO: 16 - protein, 9 aa, Homo sapiens
YLLEHVVRI

SEQ ID NO: 17 - protein, 9 aa, Homo sapiens
YALEHVVRV

SEQ ID NO: 18 - protein, 9 aa, Homo sapiens
YALEHVVRL

SEQ ID NO: 19 - protein, 9 aa, Homo sapiens
YALEHVVRA

SEQ ID NO: 20 - protein, 9 aa, Homo sapiens
YALEHVVRI

SEQ ID NO: 21 - protein, 9 aa, Homo sapiens
YVLEHVVRV

SEQ ID NO: 22 - protein, 9 aa, Homo sapiens
YVLEHVVRL

SEQ ID NO: 23 - protein, 9 aa, Homo sapiens
YVLEHVVRA

SEQ ID NO: 24 - protein, 9 aa, Homo sapiens
YVLEHVVRI

SEQ ID NO: 25 - protein, 9 aa, Homo sapiens
  misc_feature (1)..(1): Xaa can be Lys or Tyr
  misc_feature (2)..(2): Xaa can be Val, Leu or Ala
  misc_feature (9)..(9): Xaa can be Val, Leu, Ala or Ile
XXLEHVVRX

SEQ ID NO: 26 - DNA, 36 bp, Homo sapiens
ggaattccatatgagtcaacaaggagaagaagatcc

SEQ ID NO: 27 - DNA, 36 bp, Homo sapiens
ttgtcagtcgacttagagtctctcagctggtacacg

SEQ ID NO: 28 - DNA, 36 bp, Homo sapiens
tctctcatatggatggtggaattactcaatccccaa

SEQ ID NO: 29 - DNA, 32 bp, Homo sapiens
tagaaaccggtggccaggcacaccagtgtggc

SEQ ID NO: 30 - protein, 9 aa, Homo sapiens
AVLEHVVRV

SEQ ID NO: 31 - protein, 9 aa, Homo sapiens
KALEHVVRV

SEQ ID NO: 32 - protein, 9 aa, Homo sapiens
KVAEHVVRV

SEQ ID NO: 33 - protein, 9 aa, Homo sapiens
KVLAHVVRV

SEQ ID NO: 34 - protein, 9 aa, Homo sapiens
KVLEAVVRV

SEQ ID NO: 35 - protein, 9 aa, Homo sapiens
KVLEHAVRV

SEQ ID NO: 36 - protein, 9 aa, Homo sapiens
KVLEHVARV

SEQ ID NO: 37 - protein, 9 aa, Homo sapiens
KVLEHVVAV

SEQ ID NO: 38 - protein, 9 aa, Homo sapiens
KVLEHVVRA

SEQ ID NO: 39 - protein, 274 aa, Homo sapiens
MEKMLECAFIVLWLQLGWLSGEDQVTQSPEALRLQEGESSSLNCSYTVSGLRGLFWYRQDPGKGPEFLFTLYSAGEEKEKERLKATLTKKESFLHITAPKPEDSATYLCAVQGENSGYSTLTFGKGTMLLVSPDIQNPDPAVYQLRDSKSSDKSVCLFTDFDSQTNVSQSKDSDVYITDKTVLDMRSMDFKSNSAVAWSNKSDFACANAFNNSIIPEDTFFPSPESSCDVKLVEKSFETDTNLNFQNLSVIGFRILLLKVAGFNLLMTLRLWSS

SEQ ID NO: 40 - protein, 21 aa, Homo sapiens
MEKMLECAFIVLWLQLGWLSG

SEQ ID NO: 41 - protein, 112 aa, Homo sapiens
MEKMLECAFIVLWLQLGWLSGEDQVTQSPEALRLQEGESSSLNCSYTVSGLRGLFWYRQDPGKGPEFLFTLYSAGEEKEKERLKATLTKKESFLHITAPKPEDSATYLCAVQ

SEQ ID NO: 42 - protein, 6 aa, Homo sapiens
VSGLRG

SEQ ID NO: 43 - protein, 3 aa, Homo sapiens
LYS

SEQ ID NO: 44 - protein, 15 aa, Homo sapiens
CAVQGENSGYSTLTF

SEQ ID NO: 45 - protein, 19 aa, Homo sapiens
NSGYSTLTFGKGTMLLVSP

SEQ ID NO: 46 - protein, 141 aa, Homo sapiens
DIQNPDPAVYQLRDSKSSDKSVCLFTDFDSQTNVSQSKDSDVYITDKTVLDMRSMDFKSNSAVAWSNKSDFACANAFNNSIIPEDTFFPSPESSCDVKLVEKSFETDTNLNFQNLSVIGFRILLLKVAGFNLLMTLRLWSS

SEQ ID NO: 47 - protein, 314 aa, Homo sapiens
MGPQLLGYVVLCLLGAGPLEAQVTQNPRYLITVTGKKLTVTCSQNMNHEYMSWYRQDPGLGLRQIYYSMNVEVTDKGDVPEGYKVSRKEKRNFPLILESPSPNQTSLYFCASSLGPGLAAYNEQFFGPGTRLTVLEDLKNVFPPEVAVFEPSEAEISHTQKATLVCLATGFYPDHVELSWWVNGKEVHSGVSTDPQPLKEQPALNDSRYCLSSRLRVSATFWQNPRNHFRCQVQFYGLSENDEWTQDRAKPVTQIVSAEAWGRADCGFTSESYQQGVLSATILYEILLGKATLYAVLVSALVLMAMVKRKDSRG

SEQ ID NO: 48 - protein, 19 aa, Homo sapiens
MGPQLLGYVVLCLLGAGPL

SEQ ID NO: 49 - protein, 114 aa, Homo sapiens
MGPQLLGYVVLCLLGAGPLEAQVTQNPRYLITVTGKKLTVTCSQNMNHEYMSWYRQDPGLGLRQIYYSMNVEVTDKGDVPEGYKVSRKEKRNFPLILESPSPNQTSLYFCASSL

SEQ ID NO: 50 - protein, 5 aa, Homo sapiens
MNHEY

SEQ ID NO: 51 - protein, 6 aa, Homo sapiens
SMNVEV

SEQ ID NO: 52 - protein, 16 aa, Homo sapiens
CASSLGPGLAAYNEQF

SEQ ID NO: 53 - protein, 15 aa, Homo sapiens
YNEQFFGPGTRLTVL

SEQ ID NO: 54 - protein, 179 aa, Homo sapiens
EDLKNVFPPEVAVFEPSEAEISHTQKATLVCLATGFYPDHVELSWWVNGKEVHSGVSTDPQPLKEQPALNDSRYCLSSRLRVSATFWQNPRNHFRCQVQFYGLSENDEWTQDRAKPVTQIVSAEAWGRADCGFTSESYQQGVLSATILYEILLGKATLYAVLVSALVLMAMVKRKDSRG

SEQ ID NO: 55 - protein, 272 aa, Homo sapiens
MKTFAGFSFLFLWLQLDCMSRGEDVEQSLFLSVREGDSSVINCTYTDSSSTYLYWYKQEPGAGLQLLTYIFSNMDMKQDQRLTVLLNKKDKHLSLRIADTQTGDSAIYFCAEYSSASKIIFGSGTRLSIRPNIQNPDPAVYQLRDSKSSDKSVCLFTDFDSQTNVSQSKDSDVYITDKTVLDMRSMDFKSNSAVAWSNKSDFACANAFNNSIIPEDTFFPSPESSCDVKLVEKSFETDTNLNFQNLSVIGFRILLLKVAGFNLLMTLRLWSS

SEQ ID NO: 56 - protein, 21 aa, Homo sapiens
MKTFAGFSFLFLWLQLDCMSR

SEQ ID NO: 57 - protein, 112 aa, Homo sapiens
MKTFAGFSFLFLWLQLDCMSRGEDVEQSLFLSVREGDSSVINCTYTDSSSTYLYWYKQEPGAGLQLLTYIFSNMDMKQDQRLTVLLNKKDKHLSLRIADTQTGDSAIYFCAE

SEQ ID NO: 58 - protein, 6 aa, Homo sapiens
DSSSTY

SEQ ID NO: 59 - protein, 3 aa, Homo sapiens
IFS

SEQ ID NO: 60 - protein, 12 aa, Homo sapiens
CAEYSSASKIIF

SEQ ID NO: 61 - protein, 19 aa, Homo sapiens
YSSASKIIFGSGTRLSIRP

SEQ ID NO: 62 - protein, 141 aa, Homo sapiens
NIQNPDPAVYQLRDSKSSDKSVCLFTDFDSQTNVSQSKDSDVYITDKTVLDMRSMDFKSNSAVAWSNKSDFACANAFNNSIIPEDTFFPSPESSCDVKLVEKSFETDTNLNFQNLSVIGFRILLLKVAGFNLLMTLRLWSS

SEQ ID NO: 63 - protein, 310 aa, Homo sapiens
MGSWTLCCVSLCILVAKHTDAGVIQSPRHEVTEMGQEVTLRCKPISGHDYLFWYRQTMMRGLELLIYFNNNVPIDDSGMPEDRFSAKMPNASFSTLKIQPSEPRDSAVYFCASRANTGELFFGEGSRLTVLEDLKNVFPPEVAVFEPSEAEISHTQKATLVCLATGFYPDHVELSWWVNGKEVHSGVSTDPQPLKEQPALNDSRYCLSSRLRVSATFWQNPRNHFRCQVQFYGLSENDEWTQDRAKPVTQIVSAEAWGRADCGFTSESYQQGVLSATILYEILLGKATLYAVLVSALVLMAMVKRKDSRG

SEQ ID NO: 64 - protein, 19 aa, Homo sapiens
MGSWTLCCVSLCILVAKHT

SEQ ID NO: 65 - protein, 113 aa, Homo sapiens
MGSWTLCCVSLCILVAKHTDAGVIQSPRHEVTEMGQEVTLRCKPISGHDYLFWYRQTMMRGLELLIYFNNNVPIDDSGMPEDRFSAKMPNASFSTLKIQPSEPRDSAVYFCAS

SEQ ID NO: 66 - protein, 5 aa, Homo sapiens
SGHDY

SEQ ID NO: 67 - protein, 6 aa, Homo sapiens
FNNNVP

SEQ ID NO: 68 - protein, 12 aa, Homo sapiens
CASRANTGELFF

SEQ ID NO: 69 - protein, 16 aa, Homo sapiens
NTGELFFGEGSRLTVL

SEQ ID NO: 70 - protein, 179 aa, Homo sapiens; identical to SEQ ID NO: 54

SEQ ID NO: 71 - protein, 277 aa, Homo sapiens
MLTASLLRAVIASICVVSSMAQKVTQAQTEISVVEKEDVTLDCVYETRDTTYYLFWYKQPPSGELVFLIRRNSFDEQNEISGRYSWNFQKSTSSFNFTITASQVVDSAVYFCALSEGNSGNTPLVFGKGTRLSVIANIQNPDPAVYQLRDSKSSDKSVCLFTDFDSQTNVSQSKDSDVYITDKTVLDMRSMDFKSNSAVAWSNKSDFACANAFNNSIIPEDTFFPSPESSCDVKLVEKSFETDTNLNFQNLSVIGFRILLLKVAGFNLLMTLRLWSS

SEQ ID NO: 72 - protein, 20 aa, Homo sapiens
MLTASLLRAVIASICVVSSM

SEQ ID NO: 73 - protein, 116 aa, Homo sapiens
MLTASLLRAVIASICVVSSMAQKVTQAQTEISVVEKEDVTLDCVYETRDTTYYLFWYKQPPSGELVFLIRRNSFDEQNEISGRYSWNFQKSTSSFNFTITASQVVDSAVYFCALSE

SEQ ID NO: 74 - protein, 7 aa, Homo sapiens
TRDTTYY

SEQ ID NO: 75 - protein, 4 aa, Homo sapiens
RNSF

SEQ ID NO: 76 - protein, 15 aa, Homo sapiens
CALSEGNSGNTPLVF

SEQ ID NO: 77 - protein, 19 aa, Homo sapiens
NSGNTPLVFGKGTRLSVIA

SEQ ID NO: 78 - protein, 141 aa, Homo sapiens; identical to SEQ ID NO: 62

SEQ ID NO: 79 - protein, 313 aa, Homo sapiens
MGIRLLCRVAFCFLAVGLVDVKVTQSSRYLVKRTGEKVFLECVQDMDHENMFWYRQDPGLGLRLIYFSYDVKMKEKGDIPEGYSVSREKKERFSLILESASTNQTSMYLCASSLSSGSHQETQYFGPGTRLLVLEDLKNVFPPEVAVFEPSEAEISHTQKATLVCLATGFYPDHVELSWWVNGKEVHSGVSTDPQPLKEQPALNDSRYCLSSRLRVSATFWQNPRNHFRCQVQFYGLSENDEWTQDRAKPVTQIVSAEAWGRADCGFTSESYQQGVLSATILYEILLGKATLYAVLVSALVLMAMVKRKDSRG

SEQ ID NO: 80 - protein, 19 aa, Homo sapiens
MGIRLLCRVAFCFLAVGLV

SEQ ID NO: 81 - protein, 114 aa, Homo sapiens
MGIRLLCRVAFCFLAVGLVDVKVTQSSRYLVKRTGEKVFLECVQDMDHENMFWYRQDPGLGLRLIYFSYDVKMKEKGDIPEGYSVSREKKERFSLILESASTNQTSMYLCASSL

SEQ ID NO: 82 - protein, 5 aa, Homo sapiens
MDHEN

SEQ ID NO: 83 - protein, 6 aa, Homo sapiens
SYDVKM

SEQ ID NO: 84 - protein, 16 aa, Homo sapiens
CASSLSSGSHQETQYF

SEQ ID NO: 85 - protein, 15 aa, Homo sapiens
QETQYFGPGTRLLVL

SEQ ID NO: 86 - protein, 179 aa, Homo sapiens; identical to SEQ ID NO: 54

SEQ ID NO: 87 - protein, 20 aa, Homo sapiens
VIGFRILLLKVAGFNLLMTL

SEQ ID NO: 88 - protein, 23 aa, Homo sapiens
TILYEILLGKATLYAVLVSALVL

SEQ ID NO: 89 - protein, 274 aa, Homo sapiens
METLLGLLILWLQLQWVSSKQEVTQIPAALSVPEGENLVLNCSFTDSAIYNLQWFRQDPGKGLTSLLLIQSSQREQTSGRLNASLDKSSGRSTLYIAASQPGDSATYLCAVRPTSGGSYIPTFGRGTSLIVHPYIQNPDPAVYQLRDSKSSDKSVCLFTDFDSQTNVSQSKDSDVYITDKTVLDMRSMDFKSNSAVAWSNKSDFACANAFNNSIIPEDTFFPSPESSCDVKLVEKSFETDTNLNFQNLSVIGFRILLLKVAGFNLLMTLRLWSS

SEQ ID NO: 90 - protein, 311 aa, Homo sapiens
MSIGLLCCAALSLLWAGPVNAGVTQTPKFQVLKTGQSMTLQCAQDMNHEYMSWYRQDPGMGLRLIHYSVGAGITDQGEVPNGYNVSRSTTEDFPLRLLSAAPSQTSVYFCASSYVGNTGELFFGEGSRLTVLEDLKNVFPPEVAVFEPSEAEISHTQKATLVCLATGFYPDHVELSWWVNGKEVHSGVSTDPQPLKEQPALNDSRYCLSSRLRVSATFWQNPRNHFRCQVQFYGLSENDEWTQDRAKPVTQIVSAEAWGRADCGFTSESYQQGVLSATILYEILLGKATLYAVLVSALVLMAMVKRKDSRG

SEQ ID NO: 91 - protein, 9 aa, Homo sapiens
FLLETVVRV

SEQ ID NO: 92 - protein, 9 aa, Homo sapiens
ILDEHVQRV

SEQ ID NO: 93 - protein, 9 aa, Homo sapiens
IVMEHVVFL

SEQ ID NO: 94 - protein, 9 aa, Homo sapiens
KILEDVVGV

SEQ ID NO: 95 - protein, 9 aa, Homo sapiens
KLLDLQVRV

SEQ ID NO: 96 - protein, 9 aa, Homo sapiens
KVLDKVFRA

SEQ ID NO: 97 - protein, 9 aa, Homo sapiens
KVLEILHRV

SEQ ID NO: 98 - protein, 9 aa, Homo sapiens
KVLERVNAV

SEQ ID NO: 99 - protein, 9 aa, Homo sapiens
KVLETLVTV

SEQ ID NO: 100 - protein, 9 aa, Homo sapiens
KVLGIVVGV

SEQ ID NO: 101 - protein, 9 aa, Homo sapiens
SLLMWITQV